European Patent Application EP 4 458 371 A1, published November 6, 2024. Title: SUPEROXIDE DISMUTASE AND USES THEREOF FOR PREVENTING OR TREATING DRY EYE SYNDROME. Applicant: BiomLogic, Inc. GENOFOCUS CO., LTD. The sequence listing filed with the application follows.

SEQUENCE LISTING (72 sequences)

SEQ ID NO: 1 - DNA, 609 bp, Bacillus amyloliquefaciens
atggcttacaaacttccagaattgccttacgcttatgatgctttagaacctcatatcgataaggaaacgatgacgattcaccatacgaagcaccataacacatacgtgacaaacctcaacaaagcgatcgaaggatctgcgcttgcagagaaatctgtagatgagcttgttgctgatttgaacgcagtgccggaggacatccgcacggcagtccgcaacaatggcggcggacatgcaaaccactctttattctggactcttttatctccgaacggcggaggcgaaccgactggtgagcttgctgaagagatcaaaagcacgttcggaagcttcgatcaatttaaagaaaaattcgccgcagcagctgcaggccgtttcggttcaggctgggcttggctcgttgtaaacaacggcaaacttgaaattacaagcacgccaaaccaagattcaccgctttcagaaggtaaaacacctgttctcggtcttgatgtttgggagcatgcgtactacctgaactaccaaaaccgccgtcctgattacatttcagctttctggaatgttgtgaactgggatgaagttgcccgtctttacagcgaagcaaaataatga

SEQ ID NO: 2 - protein, 201 aa, Bacillus amyloliquefaciens
MAYKLPELPYAYDALEPHIDKETMTIHHTKHHNTYVTNLNKAIEGSALAEKSVDELVADLNAVPEDIRTAVRNNGGGHANHSLFWTLLSPNGGGEPTGELAEEIKSTFGSFDQFKEKFAAAAAGRFGSGWAWLVVNNGKLEITSTPNQDSPLSEGKTPVLGLDVWEHAYYLNYQNRRPDYISAFWNVVNWDEVARLYSEAK

SEQ ID NO: 3 - DNA, 609 bp, Bacillus amyloliquefaciens
atggcttacaaacttccagaattgccttacgcttatgatgctttagaacctcatatcgataaggaaacgatgacgattcaccatacgaagcaccataacacatacgtgacaaacctcaacaaagcgatcgaaggatctgcgcttgcagagaaatctgtagatgagcttgttgctgatttgaacgcagtgccggaggacatccgcacggcagtccgcaacgatggcggcggacatgcaaaccactctttattctggactcttttatctccgaacggcggaggcgaaccgactggtgagcttgctgaagagatcaaaagcacgttcggaagcttcgatcaatttaaagaaaaattcgccgcagcagctgcaggccgtttcggttcaggctgggcttggctcgttgtaaacgacggcaaacttgaaattacaagcacgccaaaccaagattcaccgctttcagaaggtaaaacacctgttctcggtcttgatgtttgggagcatgcgtactacctgaactaccaaaaccgccgtcctgattacatttcagctttctggaatgttgtgaactgggatgaagttgcccgtctttacagcgaagcaaaataatga

SEQ ID NO: 4 - protein, 201 aa, Bacillus amyloliquefaciens
MAYKLPELPYAYDALEPHIDKETMTIHHTKHHNTYVTNLNKAIEGSALAEKSVDELVADLNAVPEDIRTAVRNDGGGHANHSLFWTLLSPNGGGEPTGELAEEIKSTFGSFDQFKEKFAAAAAGRFGSGWAWLVVNDGKLEITSTPNQDSPLSEGKTPVLGLDVWEHAYYLNYQNRRPDYISAFWNVVNWDEVARLYSEAK

SEQ ID NO: 5 - DNA, 37 bp, Artificial Sequence
  aprE_frgament 1_forward primer
ctacggggtctgacgcagatatcgtaaccgaagaacg

SEQ ID NO: 6 - DNA, 28 bp, Artificial Sequence
  aprE_frgament 1_reverse primer
tgttgcagacatgttgctgaacgccatc

SEQ ID NO: 7 - DNA, 28 bp, Artificial Sequence
  aprE_frgament 2_forward primer
caacatgtctgcaacatatcttggaaac

SEQ ID NO: 8 - DNA, 38 bp, Artificial Sequence
  aprE_frgament 2_reverse
gataagctgtcaaaccagagattggataggctatcaag

SEQ ID NO: 9 - DNA, 38 bp, Artificial Sequence
  nprE_frgament 1_forward primer
ctacggggtctgacgcagggcattactgcaccataatc

SEQ ID NO: 10 - DNA, 28 bp, Artificial Sequence
  nprE_frgament 1_reverse primer
gaggtacgccttcagcagcctgaacacc

SEQ ID NO: 11 - DNA, 28 bp, Artificial Sequence
  nprE_frgament 2_forward primer
gctgaaggcgtacctcacgccttcttcc

SEQ ID NO: 12 - DNA, 38 bp, Artificial Sequence
  nprE_frgament 2_reverse primer
gataagctgtcaaaccagttgtcagatttgcatccttc

SEQ ID NO: 13 - DNA, 38 bp, Artificial Sequence
  bpr_frgament 1_forward primer
ctacggggtctgacgcagagcaatttccagcccgcttc

SEQ ID NO: 14 - DNA, 28 bp, Artificial Sequence
  bpr_frgament 1_reverse primer
gtatgatgaggcatgaacagcaatcccg

SEQ ID NO: 15 - DNA, 28 bp, Artificial Sequence
  bpr_frgament 2_forward primer
tcatgcctcatcatactcaacaagggtg

SEQ ID NO: 16 - DNA, 38 bp, Artificial Sequence
  bpr_frgament 2_reverse primer
gataagctgtcaaaccagttcccagccggatgttcaac

SEQ ID NO: 17 - DNA, 38 bp, Artificial Sequence
  epr_frgament 1_forward primer
ctacggggtctgacgcaggctttctgccagccgatagg

SEQ ID NO: 18 - DNA, 28 bp, Artificial Sequence
  epr_frgament 1_reverse primer
tgtgtcaaagccgttatgcttggctccg

SEQ ID NO: 19 - DNA, 28 bp, Artificial Sequence
  epr_frgament 2_forward primer
taacggctttgacacagcacaaactgcc

SEQ ID NO: 20 - DNA, 38 bp, Artificial Sequence
  epr_frgament 2_reverse primer
gataagctgtcaaaccaggtctcccatacatgaacgac

SEQ ID NO: 21 - DNA, 38 bp, Artificial Sequence
  nprB_frgament 1_forward primer
ctacggggtctgacgcagagtaatcttgtaggaggctg

SEQ ID NO: 22 - DNA, 28 bp, Artificial Sequence
  nprB_frgament 1_reverse primer
tgtgactgtcatattcaccgtcgtgtgg

SEQ ID NO: 23 - DNA, 29 bp, Artificial Sequence
  nprB_frgament 2_forward primer
tgaatatgacagtcacacagtattccgcc

SEQ ID NO: 24 - DNA, 38 bp, Artificial Sequence
  nprB_frgament 2_reverse primer
gataagctgtcaaaccagattaggatacggtctggctg

SEQ ID NO: 25 - DNA, 38 bp, Artificial Sequence
  vpr_frgament 1_forward primer
ctacggggtctgacgcagatgtacgctgagccgaatag

SEQ ID NO: 26 - DNA, 28 bp, Artificial Sequence
  vpr_frgament 1_reverse primer
ggaatcacatttgcggagatacggcgtc

SEQ ID NO: 27 - DNA, 28 bp, Artificial Sequence
  vpr_frgament 2_forward primer
ccgcaaatgtgattccggcacatcaaac

SEQ ID NO: 28 - DNA, 38 bp, Artificial Sequence
  vpr_frgament 2_reverse primer
gataagctgtcaaaccagaccgttttccgaatctgacc

SEQ ID NO: 29 - DNA, 38 bp, Artificial Sequence
  mpr_frgament 1_forward primer
ctacggggtctgacgcagcgttatcccgaatgcccgtg

SEQ ID NO: 30 - DNA, 28 bp, Artificial Sequence
  mpr_frgament 1_reverse primer
ggctttgttcctttagtgtcaaccaccc

SEQ ID NO: 31 - DNA, 28 bp, Artificial Sequence
  mpr_frgament 2_forward primer
ctaaaggaacaaagccgattcgctccgc

SEQ ID NO: 32 - DNA, 38 bp, Artificial Sequence
  mpr_frgament 2_reverse primer
gataagctgtcaaaccagaaattgactgctccacgctg

SEQ ID NO: 33 - DNA, 38 bp, Artificial Sequence
  srfAC_frgament 1_forward primer
ctacggggtctgacgcaggatatgtattacctatcgcc

SEQ ID NO: 34 - DNA, 29 bp, Artificial Sequence
  srfAC_frgament 1_reverse primer
gccccttcatccagttcactgcttccttg

SEQ ID NO: 35 - DNA, 33 bp, Artificial Sequence
  srfAC_frgament 2_forward primer
ggaagcagtgaactggatgaaggggcttcgctg

SEQ ID NO: 36 - DNA, 38 bp, Artificial Sequence
  srfAC_frgament 2_reverse primer
gataagctgtcaaaccagaacgcttcgacatcactttc

SEQ ID NO: 37 - DNA, 38 bp, Artificial Sequence
  spoIIA_frgament 1_forward primer
ctacggggtctgacgcagagcggacgatgggagactgg

SEQ ID NO: 38 - DNA, 28 bp, Artificial Sequence
  spoIIA_frgament 1_reverse primer
gccacctcatgcagccgatctggaagag

SEQ ID NO: 39 - DNA, 28 bp, Artificial Sequence
  spoIIA_frgament 2_forward primer
ggctgcatgaggtggctgagcggctcgg

SEQ ID NO: 40 - DNA, 38 bp, Artificial Sequence
  spoIIA_frgament 2_reverse primer
gataagctgtcaaaccagctcattgttttggtgagctg

SEQ ID NO: 41 - DNA, 38 bp, Artificial Sequence
  ispA_frgament 1_forward primer
ctacggggtctgacgcagtgctgcttggcattcatttc

SEQ ID NO: 42 - DNA, 29 bp, Artificial Sequence
  ispA_frgament 1_reverse primer
gccattgaagcaatgcctccgtttgaatc

SEQ ID NO: 43 - DNA, 33 bp, Artificial Sequence
  ispA_frgament 2_forward primer
acggaggcattgcttcaatggctgcccctcatg

SEQ ID NO: 44 - DNA, 38 bp, Artificial Sequence
  ispA_frgament 2_reverse primer
gataagctgtcaaaccagtcaatgctctcgtcatattc

SEQ ID NO: 45 - DNA, 38 bp, Artificial Sequence
  epsE_frgament 1_forward primer
ctacggggtctgacgcagcaagcaaatgggctgggagg

SEQ ID NO: 46 - DNA, 28 bp, Artificial Sequence
  epsE_frgament 1_reverse primer
gacaagccatgctttctgccaaagtgcg

SEQ ID NO: 47 - DNA, 28 bp, Artificial Sequence
  epsE_frgament 2_forward primer
gaaagcatggcttgtcaagcatgaatag

SEQ ID NO: 48 - DNA, 38 bp, Artificial Sequence
  epsE_frgament 2_reverse primer
gataagctgtcaaaccagtgttgtatacattcagcagc

SEQ ID NO: 49 - DNA, 29 bp, Artificial Sequence
  xpf_frgament 1_forward primer
gatcctctacggttcatccatgtccgaac

SEQ ID NO: 50 - DNA, 22 bp, Artificial Sequence
  xpf_frgament 1_reverse primer
tctatgatcctcctcatttttg

SEQ ID NO: 51 - DNA, 35 bp, Artificial Sequence
  xpf_frgament 2_forward primer
gaggaggatcatagaaagcttgtcatacgtttgcc

SEQ ID NO: 52 - DNA, 33 bp, Artificial Sequence
  xpf_frgament 2_reverse primer
gagttttcgttcggatcctccgctttttgtttg

SEQ ID NO: 53 - DNA, 20 bp, Artificial Sequence
  AprE_PCR primer_forward
caaggcttgaaataacgttg

SEQ ID NO: 54 - DNA, 20 bp, Artificial Sequence
  AprE_PCR primer_reverse
ttcgctgattacaacattgg

SEQ ID NO: 55 - DNA, 20 bp, Artificial Sequence
  NprE_PCR primer_forward
ggaacagatgatagctcatc

SEQ ID NO: 56 - DNA, 20 bp, Artificial Sequence
  NprE_PCR primer_reverse
acactccgagaaggctgaag

SEQ ID NO: 57 - DNA, 20 bp, Artificial Sequence
  Vpr_PCR primer_forward
ctgcggcctgcacagccgcc

SEQ ID NO: 58 - DNA, 20 bp, Artificial Sequence
  Vpr_PCR primer_reverse
cgctgaatgacggtggtaag

SEQ ID NO: 59 - DNA, 20 bp, Artificial Sequence
  NprB_PCR primer_forward
agtaatcttgtaggaggctg

SEQ ID NO: 60 - DNA, 20 bp, Artificial Sequence
  NprB_PCR primer_reverse
cgccaatgaagtgaaggagg

SEQ ID NO: 61 - DNA, 20 bp, Artificial Sequence
  Mpr_PCR primer_forward
ggttgaggcgattgcgacgg

SEQ ID NO: 62 - DNA, 20 bp, Artificial Sequence
  Mpr_PCR primer_reverse
ccattctgcaaaatcagctc

SEQ ID NO: 63 - DNA, 20 bp, Artificial Sequence
  spoIIAC_PCR primer_forward
aagatatgaagaaagccggg

SEQ ID NO: 64 - DNA, 20 bp, Artificial Sequence
  spoIIAC_PCR primer_reverse
acagccgcttcataagcctg

SEQ ID NO: 65 - DNA, 20 bp, Artificial Sequence
  ThrC_PCR primer_forward
tcaagctgtcatgtacggag

SEQ ID NO: 66 - DNA, 20 bp, Artificial Sequence
  ThrC_PCR primer_reverse
tccgatacgaatggctgtcg

SEQ ID NO: 67 - DNA, 23 bp, Artificial Sequence
  SOD_forward primer
ggaggaattacaatggcttacaa

SEQ ID NO: 68 - DNA, 27 bp, Artificial Sequence
  D74_reverse primer
tgcatgtccgccgccatcgttgcggac

SEQ ID NO: 69 - DNA, 27 bp, Artificial Sequence
  D74_forward primer
cagtccgcaacgatggcggcggacatg

SEQ ID NO: 70 - DNA, 28 bp, Artificial Sequence
  D137_reverse primer
ttcaagtttgccgtcgtttacaacgagc

SEQ ID NO: 71 - DNA, 25 bp, Artificial Sequence
  D137_forward primer
ctcgttgtaaacgacggcaaacttg

SEQ ID NO: 72 - DNA, 26 bp, Artificial Sequence
  SOD_reverse primer
caaaacagaagcttcattattttgct